European Patent Specification EP 3 548 512 B1, published August 2, 2023. Title: USE OF PEPTIDE COMPOUNDS FOR PROMOTING SURVIVAL, GROWTH AND CELL DIFFERENTIATION. Applicant: NEURONAX. The sequence listing filed with the application follows.

SEQUENCE LISTING (37 sequences)

SEQ ID NO: 1 - protein, 9 aa, Artificial Sequence
  Peptide compound
  misc_feature (1)..(1): X is W or L-Nal2
  misc_feature (3)..(3): X is G, V, A, S or Abu
  misc_feature (6)..(6): X is S, D or A
  misc_feature (7)..(7): X is C or Abu wherein the cysteine residue can be inked to the cysteine residue of X in position 9 by a disulfide bond
  misc_feature (9)..(9): X is R-S, R-S-Nm, R-S-C-G, R-Abu-Nm, R-Abu-C-G, K-iPr-S-Nm or K-iPr-S-C-G wherein the cysteine residue can be linked to the cysteine residue of X in position 7 by a disulfide bond
XSXWSXXSX

SEQ ID NO: 2 - protein, 9 aa, Artificial Sequence
  Peptide compound
  MISC_FEATURE (1)..(1): X is W or L-Nal2
  MISC_FEATURE (3)..(3): X is G
  MISC_FEATURE (6)..(6): X is S
  MISC_FEATURE (7)..(7): X is C or Abu wherein the cysteine residue can be linked to the cysteine residue of X in position 9 by a disulfide bond
  MISC_FEATURE (9)..(9): X is R-S, R-S-Nm, R-S-C-G, R-Abu-Nm, R-Abu-C-G, K-iPr-S-Nm or K-iPr-S-C-G wherein the cysteine residue can be linked to the cysteine residue of X in position 7 by a disulfide bond
XSXWSXXSX

SEQ ID NO: 3 - protein, 10 aa, Artificial Sequence
  Peptide compound
  misc_feature (7)..(7): X is C or Abu
WSGWSSXSRS

SEQ ID NO: 4 - protein, 10 aa, Artificial Sequence
  Peptide compound
WSGWSSCSRS

SEQ ID NO: 5 - protein, 10 aa, Artificial Sequence
  Peptide compound
  misc_feature (9)..(9): the COOH end has been replaced by a NH2 end
WSGWSSCSRS

SEQ ID NO: 6 - protein, 12 aa, Artificial Sequence
  Peptide compound
WSGWSSCSRSCG

SEQ ID NO: 7 - protein, 12 aa, Artificial Sequence
  Peptide compound
  DISULFID (7)..(7): the cysteine residue in position 7 is linked to the cysteine residue in position 11 by a disulfide bond
  DISULFID (11)..(11): the cysteine residue in position 11 is linked to the cysteine residue in position 7 by a disulfide bond
WSGWSSCSRSCG

SEQ ID NO: 8 - protein, 10 aa, Artificial Sequence
  Peptide compound
  misc_feature (10)..(10): X is Abu the COOH end has been replaced by a NH2 end
WSGWSSCSRX

SEQ ID NO: 9 - protein, 12 aa, Artificial Sequence
  Peptide compound
  misc_feature (10)..(10): X is Abu
WSGWSSCSRXCG

SEQ ID NO: 10 - protein, 12 aa, Artificial Sequence
  Peptide compound
  DISULFID (7)..(7): the cysteine residue in position 7 is linked to the cysteine residue in position 11 by a disulfide bond
  MISC_FEATURE (10)..(10): X is Abu
  DISULFID (11)..(11): the cysteine residue in position 11 is linked to the cysteine residue in position 7 by a disulfide bond
WSGWSSCSRXCG

SEQ ID NO: 11 - protein, 11 aa, Artificial Sequence
  Peptide compound
  misc_feature (10)..(10): X is iPr
  misc_feature (11)..(11): the CCOH end has been replaced by a NH2 end
WSGWSSCSKXS

SEQ ID NO: 12 - protein, 13 aa, Artificial Sequence
  Peptide compound
  misc_feature (10)..(10): X is iPr
WSGWSSCSKXSCG

SEQ ID NO: 13 - protein, 13 aa, Artificial Sequence
  Peptide compound
  DISULFID (7)..(7): the cysteine residue in position 7 is linked to the cysteine residue in position 12 by a disulfide bond
  MISC_FEATURE (10)..(10): X is iPr
  DISULFID (12)..(12): the cysteine residue in position 12 is linked to the cysteine residue in position 7 by a disulfide bond
WSGWSSCSKXSCG

SEQ ID NO: 14 - protein, 10 aa, Artificial Sequence
  Peptide compound
  misc_feature (7)..(7): X is Abu
WSGWSSXSRS

SEQ ID NO: 15 - protein, 10 aa, Artificial Sequence
  Peptide compound
  misc_feature (7)..(7): X is Abu
  misc_feature (10)..(10): the COOH end has been replaced by a NH2 end
WSGWSSXSRS

SEQ ID NO: 16 - protein, 12 aa, Artificial Sequence
  Peptide compound
  misc_feature (7)..(7): X is Abu
WSGWSSXSRSCG

SEQ ID NO: 17 - protein, 10 aa, Artificial Sequence
  Peptide compound
  misc_feature (7)..(7): X is Abu
  misc_feature (10)..(10): X is Abu the COOH end has been replaced by a NH2 end
WSGWSSXSRX

SEQ ID NO: 18 - protein, 12 aa, Artificial Sequence
  Peptide compound
  misc_feature (7)..(7): X is Abu
  misc_feature (10)..(10): X is Abu
WSGWSSXSRXCG

SEQ ID NO: 19 - protein, 11 aa, Artificial Sequence
  Peptide compound
  misc_feature (7)..(7): X is Abu
  misc_feature (10)..(10): X is iPr
  misc_feature (11)..(11): the COOH end has been replaced y a NH2 end
WSGWSSXSKXS

SEQ ID NO: 20 - protein, 13 aa, Artificial Sequence
  Peptide compound
  misc_feature (7)..(7): X is Abu
  misc_feature (10)..(10): X is iPr
WSGWSSXSKXSCG

SEQ ID NO: 21 - protein, 10 aa, Artificial Sequence
  Peptide compound
  misc_feature (1)..(1): X is L-Nal2
XSGWSSCSRS

SEQ ID NO: 22 - protein, 10 aa, Artificial Sequence
  Peptide compound
  misc_feature (1)..(1): X is L-Nal2
  misc_feature (10)..(10): the COOH end has been replaced by a NH2 end
XSGWSSCSRS

SEQ ID NO: 23 - protein, 12 aa, Artificial Sequence
  Peptide compound
  misc_feature (1)..(1): X is L-Nal2
XSGWSSCSRSCG

SEQ ID NO: 24 - protein, 12 aa, Artificial Sequence
  Peptide compound
  misc_feature (1)..(1): X is L-Nal2
  DISULFID (7)..(7): the cysteine residue in position 7 is linked to the cysteine residue in position 11 by a disulfide bond
  DISULFID (11)..(11): the cysteine residue in position 11 is linked to the cysteine residue in position 7 by a disulfide bond
XSGWSSCSRSCG

SEQ ID NO: 25 - protein, 10 aa, Artificial Sequence
  Peptide compound
  misc_feature (1)..(1): X is L-Nal2
  misc_feature (10)..(10): X is Abu the COOH end has been replaced by a NH2 end
XSGWSSCSRX

SEQ ID NO: 26 - protein, 12 aa, Artificial Sequence
  Peptide compound
  misc_feature (1)..(1): X is L-Nal2
  misc_feature (10)..(10): X is Abu
XSGWSSCSRXCG

SEQ ID NO: 27 - protein, 12 aa, Artificial Sequence
  Peptide compound
  misc_feature (1)..(1): X is L-Nal2
  DISULFID (7)..(7): the cysteine residue in position 7 is linked to the cysteine residue in position 11 by a disulfide bond
  MISC_FEATURE (10)..(10): X is Abu
  DISULFID (11)..(11): the cysteine residue in position 11 is linked to the cysteine residue in position 7 by a disulfide bond
XSGWSSCSRXCG

SEQ ID NO: 28 - protein, 11 aa, Artificial Sequence
  Peptide compound
  misc_feature (1)..(1): X is L-Nal2
  misc_feature (10)..(10): X is iPr
  misc_feature (11)..(11): the COOH end has been replaced by a NH2 end
XSGWSSCSKXS

SEQ ID NO: 29 - protein, 13 aa, Artificial Sequence
  Peptide compound
  misc_feature (1)..(1): X is L-Nal2
  misc_feature (10)..(10): X is iPr
XSGWSSCSKXSCG

SEQ ID NO: 30 - protein, 13 aa, Artificial Sequence
  Peptide compound
  misc_feature (1)..(1): X is L-Nal2
  DISULFID (7)..(7): the cysteine residue in position 7 is linked to the cysteine residue in position 12 by a disulfide bond
  misc_feature (10)..(10): X is iPr
  DISULFID (12)..(12): the cysteine residue in position 12 is linked to the cysteine residue in position 7 by a disulfide bond
XSGWSSCSKXSCG

SEQ ID NO: 31 - protein, 10 aa, Artificial Sequence
  Peptide compound
  misc_feature (1)..(1): X is L-Nal2
  misc_feature (7)..(7): X is Abu
XSGWSSXSRS

SEQ ID NO: 32 - protein, 10 aa, Artificial Sequence
  Peptide compound
  misc_feature (1)..(1): X is L-Nal2
  misc_feature (7)..(7): X is Abu
  misc_feature (10)..(10): the COOH end has been replaced by a NH2 end
XSGWSSXSRS

SEQ ID NO: 33 - protein, 12 aa, Artificial Sequence
  Peptide compound
  misc_feature (1)..(1): X is L-Nal2
  misc_feature (7)..(7): X is Abu
XSGWSSXSRSCG

SEQ ID NO: 34 - protein, 10 aa, Artificial Sequence
  Peptide compound
  misc_feature (1)..(1): X is L-Nal2
  misc_feature (7)..(7): X is Abu
  misc_feature (10)..(10): X is Abu the COOH end has been replaced by a NH2 end
XSGWSSXSRX

SEQ ID NO: 35 - protein, 12 aa, Artificial Sequence
  Peptide compound
  misc_feature (1)..(1): X is L-Nal2
  misc_feature (7)..(7): X is Abu
  misc_feature (10)..(10): X is Abu
XSGWSSXSRXCG

SEQ ID NO: 36 - protein, 11 aa, Artificial Sequence
  Peptide compound
  misc_feature (1)..(1): X is L-Nal2
  misc_feature (7)..(7): X is Abu
  misc_feature (10)..(10): X is iPr
  misc_feature (11)..(11): the COOH end has been replaced a NH2 end
XSGWSSXSKXS

SEQ ID NO: 37 - protein, 13 aa, Artificial Sequence
  Peptide compound
  misc_feature (1)..(1): X is L-Nal2
  misc_feature (7)..(7): X is Abu
  misc_feature (10)..(10): X is iPr
XSGWSSXSKXSCG